European Patent Specification EP 2 871 959 B1, published September 4, 2024. Title: METHODS FPR MODULATING PLANT RESPONSE TO ENVIRONMENTALLY-INDUCED STRESS. Applicant: HOWARD UNIVERSITY. Application PCT/US13/32496. The sequence listing filed with the application follows.

SEQUENCE LISTING (2 sequences)

SEQ ID NO: 1 - DNA, 1259 bp, Arabidopsis thaliana
ttctttgtatttccgcctcccccgagaaaacgaaaaccctagtttcagaggcatctccagacaccgaaaatggcggaaggactcgttttgaagggcaccatgcgtgcacacactgacatggtgacggcaatcgccaccccaatcgataacgcagacatcatcgtctcagcttcccgcgacaaatccatcattttgtggaaactcaccaaggacgacaaagcctacggtgtagctcagaggcgtctcactggtcactctcacttcgttgaggatgttgttctctcctccgatggacaattcgcgctttccggcagctgggacggcgagctccgtctttgggatcttgctgctggtgtctccactcgtagattcgttggacacaccaaggacgtgctctccgtcgccttctcactcgacaaccgtcagatcgtctctgcatctcgtgaccgtacgatcaagctgtggaacactcttggtgagtgcaagtacaccatttcagaaggtggtgagggacaccgtgattgggttagctgcgtcagattcagccctaacacgcttcagccgacgattgtatctgcttcgtgggacaagaccgtgaaagtgtggaacctttcgaactgcaagctcagatcgactcttgctggtcacaccggttacgtgagcactgtggctgtatcacctgatggttctctttgtgcaagtggaggcaaagacggtgttgttttgctgtgggatttggctgaggggaagaagctttactctcttgaagctaactctgtgatccatgctctttgcttcagtcccaacaggtactggctctgtgctgcaactgaacatggtattaagatttgggaccttgagagcaagagcattgttgaggatttgaaggttgatctcaaggctgaggctgaaaaggctgacaacagtggtcctgctgccaccaagaggaaggttatttactgcacaagccttaactggagcgctgatggaagcaccctcttcagtggttacaccgatggagtcattagagtttggggtattggtcgttactagtaatctcatcacttgtgctgtcgttgctctctgctatctgcttgttggttttatctatcacttatgtttttatcgacaactcatgaagtaccttgaggtttttggaaggatgtttgttttcttgtcaatctaggtttttgcttctttatcttatcgttcgagatcttggtttttagagttacttctcccgaaaaaaaaaaaaaaaa

SEQ ID NO: 2 - protein, 327 aa, Arabidopsis thaliana
MAEGLVLKGTMRAHTDMVTAIATPIDNADIIVSASRDKSIILWKLTKDDKAYGVAQRRLTGHSHFVEDVVLSSDGQFALSGSWDGELRLWDLAAGVSTRRFVGHTKDVLSVAFSLDNRQIVSASRDRTIKLWNTLGECKYTISEGGEGHRDWVSCVRFSPNTLQPTIVSASWDKTVKVWNLSNCKLRSTLAGHTGYVSTVAVSPDGSLCASGGKDGVVLLWDLAEGKKLYSLEANSVIHALCFSPNRYWLCAATEHGIKIWDLESKSIVEDLKVDLKAEAEKADNSGPAATKRKVIYCTSLNWSADGSTLFSGYTDGVIRVWGIGRY